European Patent Application EP 4 265 276 A1, published October 25, 2023. Title: Composition for Preventing or Treating Pancreatic Cancer Comprising Peptide Nucleic Acid Complex. Applicant: SEASUN THERAPEUTICS, Inc. The sequence listing filed with the application follows.

SEQUENCE LISTING (20 sequences)

SEQ ID NO: 1 - DNA, 16 bp, Artificial Sequence
  bioactive 1
acttgcttcctgtagg

SEQ ID NO: 2 - DNA, 15 bp, Artificial Sequence
  bioactive 2
agtcttgacttattg

SEQ ID NO: 3 - DNA, 16 bp, Artificial Sequence
  carrier 1
tgaacgaaggacatcc

SEQ ID NO: 4 - DNA, 16 bp, Artificial Sequence
  carrier 2
cctacaggaagcaagt

SEQ ID NO: 5 - DNA, 5 bp, Artificial Sequence
  carrier 3
catcc

SEQ ID NO: 6 - DNA, 5 bp, Artificial Sequence
  carrier 4
cctac

SEQ ID NO: 7 - DNA, 15 bp, Artificial Sequence
  carrier 5
tcagaactgaataac

SEQ ID NO: 8 - DNA, 15 bp, Artificial Sequence
  bioactive 3
atcagctccaactac

SEQ ID NO: 9 - DNA, 15 bp, Artificial Sequence
  bioactive 4
cctacgccaacagct

SEQ ID NO: 10 - DNA, 15 bp, Artificial Sequence
  bioactive 5
actccgcaattacca

SEQ ID NO: 11 - DNA, 15 bp, Artificial Sequence
  carrier 6
tagtcgaggttgatg

SEQ ID NO: 12 - DNA, 15 bp, Artificial Sequence
  carrier 7
gtagttggagctgat

SEQ ID NO: 13 - DNA, 5 bp, Artificial Sequence
  carrier 8
tgatg

SEQ ID NO: 14 - DNA, 5 bp, Artificial Sequence
  carrier 9
gtagt

SEQ ID NO: 15 - DNA, 15 bp, Artificial Sequence
  carrier 10
ggatgcggttgtcga

SEQ ID NO: 16 - DNA, 15 bp, Artificial Sequence
  carrier 11
agctgttggcgtagg

SEQ ID NO: 17 - DNA, 5 bp, Artificial Sequence
  carrier 12
gtcga

SEQ ID NO: 18 - DNA, 5 bp, Artificial Sequence
  carrier 13
agctg

SEQ ID NO: 19 - DNA, 15 bp, Artificial Sequence
  carrier 14
tgaggcgttaatggt

SEQ ID NO: 20 - protein, 13 aa, Artificial Sequence
  endosome escaper
GLFDIIKKIAESF